European Patent Application EP 4 474 375 A1, published December 11, 2024. Title: Production method of dicarboxylic acid compounds and/or diamine compounds using polyamide as a raw material. Applicant: 旭化成株式会社. The sequence listing filed with the application follows.

SEQUENCE LISTING (6 sequences)

SEQ ID NO: 1 - protein, 392 aa, Arthrobacter sp. K172
MNARSTGQHPARYPGAAAGEPTLDSWQEAPHNRWAFARLGELLPTAAVSRRDPATPAEPVVRLDALATRLPDLEQRLEETCTDAFLVLRGSEVLAEYYRAGFAPDDRHLLMSVSKSLCGTVVGALIDEGRIDPAQPVTEYVPELAGSVYDGPSVLQVLDMQISIDYNEDYVDPASEVQTHDRSAGWRTRRDGDPADTYEFLTTLRGDGGTGEFQYCSANTDVLAWIVERVTGLRYVEALSTYLWAKLDADRDATITVDQTGFGFANGGVSCTARDLARVGRMMLDGGVAPGGRVVSQGWVESVLAGGSREAMTDEGFTSAFPEGSYTRQWWCTGNERGNVSGIGIHGQNLWLDPRTDSVIVKLSSWPDPDTRHWHGLQSGILLDVSRALDAV

SEQ ID NO: 2 - protein, 355 aa, synthetic construct
  REGION 1..355: note = Arthrobacter sp. K172 NylC(m)
MNTTPVHALTDIDGGIAVDPAPRLAGPPVFGGPGNAAFDLAPVRSTGREMLRFDFPGVSIGAAHYEEGPTGATVIHIPAGARTAVDARGGAVGLSGGYDFNHAICLAGGAGYGLEAGAGVSGALLERLEYRTGFAELQLVSSAVIYDFSARSTAVYPDKALGRAALEFAVPGEFPQGRAGAGMSASAGKVDWDRTEITGQGAAFRRLGDVRILAVVVPNPVGVIVDRAGTVVRGNYDAQTGVRRHPVFDYQEAFAEQVPPVTQAGNTTISAIVTNVRMSPVELNQFAKQVHSSMHRGIQPFHTDMDGDTLFAVTTDEIDLPTTPGSSRGRLSVNATALGAIASEVMWDAVLEAGK

SEQ ID NO: 3 - DNA, 1209 bp, synthetic construct
  misc_feature 1..1209: note = Arthrobacter sp. K172 NylB
  source 1..1209: mol_type = other DNA
ataaggagatataccatgaatgcccgctctactggtcagcatccggcccggtatccgggtgcggcagcaggcgaaccaacactggactcatggcaggaagcgccccataatcgctgggcgtttgcacgcttaggcgaactgctgccaaccgctgccgtatcacgccgtgatccggcgacccctgctgaaccggtagtgcgccttgatgcgctggccactcgcttaccagacctggagcaacggctggaggaaacctgtacggatgcgttcttggttctgcgtggtagcgaagtgttagcggagtattatcgtgcaggctttgcgccggatgatcgtcacttactgatgagcgtgagcaaatcgctgtgcggaacggtcgttggagcgctgattgacgaagggcgcattgatcccgcgcaaccggtaaccgagtatgtgccggaactggccggttccgtgtatgacggcccgagtgttctccaagtccttgatatgcagatctcgatcgactacaacgaagattacgtggacccagcctcggaggttcagacccatgaccgcagtgccggatggcgtacgcgtcgtgatggcgatccggctgatacctacgagttcctgaccactttgcgcggtgacggtggtaccggtgaattccagtactgctctgcgaacacggatgttctcgcgtggattgtggagcgcgttaccgggctgcgttatgtcgaagccctcagcacatacctctgggcaaaacttgacgcagatcgggacgccactatcaccgtggatcaaaccggctttggctttgcgaatggcggggtaagttgcactgctcgtgatctggcccgcgtaggccgcatgatgctggatggcggtgtggcacctggcggtcgtgttgtctcacaagggtgggtggaatccgtcttagctggcggttctcgtgaagcgatgaccgatgaaggcttcacgtccgcctttccggaaggctcctatacgcgccagtggtggtgtacaggcaatgaacgcgggaacgtttcgggtatcggaattcacggtcagaacctgtggctggatccgcgcacagacagcgtgattgtcaagctgagcagttggcccgatcctgacacgcgccactggcatgggcttcagtctggcattttgctggatgtgagccgtgcattggatgctgtctaaaagcttgcggccgca

SEQ ID NO: 4 - DNA, 1098 bp, synthetic construct
  misc_feature 1..1098: note = Arthrobacter sp. K172 NylC(m)
  source 1..1098: mol_type = other DNA
ataaggagatataccatgaacacgacgcctgtgcatgcgcttacggacatcgatggaggcattgccgtcgatccggctccacgcctggccgggccaccggtgtttggcggtccgggcaatgcagcgtttgacctggcaccggttcgctccacgggtcgggaaatgctgcgctttgatttcccgggcgtgtctattggcgcggcccattatgaggagggtccaactggcgccactgttatccacattccagcgggtgcgcgtaccgcagttgatgcacgtggaggggcagtagggttatcgggcggctatgacttcaaccacgcaatctgcctggcgggaggtgccgggtatggacttgaagcgggagcaggcgtgagtggtgctttgttggaacggctggaatatcgcaccggctttgcggaactgcagctggtgtcgtctgcggttatctacgactttagcgcacgcagcacggcagtctatccggacaaagccttagggcgtgcggccctcgaattcgcggttcccggtgagtttccgcaaggccgtgcgggtgccggcatgagtgcgtcagcagggaaggtcgattgggatcgcaccgagattaccggccaaggcgctgcgtttcgccgcttaggcgatgtacgcattttggcggtagtcgtccccaatccggttggtgtcattgttgaccgtgctggcactgtggttcgtggcaactacgatgctcagacaggtgttcgtcgccatccggtattcgattaccaggaagccttcgccgaacaggtgccgcctgtcacacaagccggtaataccacgattagcgcaatcgtgactaacgtccgcatgagccctgtggaactgaaccagtttgccaaacaggtgcattcgtccatgcatcgtggcatccagcccttccacaccgatatggacggtgataccctgtttgctgtgaccaccgatgagattgatctgccgaccacaccggggagtagccgtggtcgcctctcagtgaatgcgaccgctctgggtgcgattgcctccgaagtgatgtgggacgcggtactggaagctggtaaataaaagcttgcggccgca

SEQ ID NO: 5 - DNA, 25 bp, synthetic construct
  misc_feature 1..25: note = primer
  source 1..25: mol_type = other DNA
aagcttgcggccgcataatgcttaa

SEQ ID NO: 6 - DNA, 35 bp, synthetic construct
  misc_feature 1..35: note = primer
  source 1..35: mol_type = other DNA
catggtatatctccttattaaagttaaacaaaatt